European Patent Specification EP 3 456 847 B1, published December 25, 2024. Title: MONITORING HEALTH AND DISEASE STATUS USING CLONOTYPE PROFILES. Applicant: Adaptive Biotechnologies Corporation. The sequence listing filed with the application follows.

SEQUENCE LISTING (197 sequences)

SEQ ID NO: 1 - DNA, 20 bp, Homo sapiens
agcgacctcgggtgggaaca

SEQ ID NO: 2 - DNA, 23 bp, Homo sapiens
aactatgttttggtatcgtcagt

SEQ ID NO: 3 - DNA, 23 bp, Homo sapiens
aactatgttttggtatcgtcagt

SEQ ID NO: 4 - DNA, 21 bp, Homo sapiens
agtgtatcctggtaccaacag

SEQ ID NO: 5 - DNA, 21 bp, Homo sapiens
agtgtgtactggtaccaacag

SEQ ID NO: 6 - DNA, 21 bp, Homo sapiens
actgtgtcctggtaccaacag

SEQ ID NO: 7 - DNA, 21 bp, Homo sapiens
agtgtgtcctggtaccaacag

SEQ ID NO: 8 - DNA, 21 bp, Homo sapiens
tctgtgtactggtaccaacag

SEQ ID NO: 9 - DNA, 20 bp, Homo sapiens
ccctttactggtaccgacag

SEQ ID NO: 10 - DNA, 20 bp, Homo sapiens
gcctttactggtaccgacag

SEQ ID NO: 11 - DNA, 21 bp, Homo sapiens
ccctttactggtaccgacaaa

SEQ ID NO: 12 - DNA, 19 bp, Homo sapiens
ttttggtaccaacaggtcc

SEQ ID NO: 13 - DNA, 19 bp, Homo sapiens
ttttggtaccaacaggccc

SEQ ID NO: 14 - DNA, 22 bp, Homo sapiens
aaccctttattggtatcaacag

SEQ ID NO: 15 - DNA, 21 bp, Homo sapiens
cgctatgtattggtacaagca

SEQ ID NO: 16 - DNA, 21 bp, Homo sapiens
cgctatgtattggtacaagca

SEQ ID NO: 17 - DNA, 23 bp, Homo sapiens
tttctggtacagacagaccatga

SEQ ID NO: 18 - DNA, 27 bp, Homo sapiens
tactatgtattggtataaacaggactc

SEQ ID NO: 19 - DNA, 22 bp, Homo sapiens
caaaatgtactggtatcaacaa

SEQ ID NO: 20 - DNA, 22 bp, Homo sapiens
caaaatgtactggtatcaacaa

SEQ ID NO: 21 - DNA, 22 bp, Homo sapiens
atgtactggtatcgacaagacc

SEQ ID NO: 22 - DNA, 23 bp, Homo sapiens
tgccatgtactggtatagacaag

SEQ ID NO: 23 - DNA, 23 bp, Homo sapiens
atacttgtcctggtatcgacaag

SEQ ID NO: 24 - DNA, 22 bp, Homo sapiens
atatgttctggtatcgacaaga

SEQ ID NO: 25 - DNA, 22 bp, Homo sapiens
atatgtcctggtatcgacaaga

SEQ ID NO: 26 - DNA, 22 bp, Homo sapiens
acatgtcctggtatcgacaaga

SEQ ID NO: 27 - DNA, 24 bp, Homo sapiens
taatctttattggtatcgacgtgt

SEQ ID NO: 28 - DNA, 20 bp, Homo sapiens
gccatgtactggtaccgaca

SEQ ID NO: 29 - DNA, 22 bp, Homo sapiens
tcatgtttactggtatcggcag

SEQ ID NO: 30 - DNA, 21 bp, Homo sapiens
caacctatactggtaccgaca

SEQ ID NO: 31 - DNA, 22 bp, Homo sapiens
catgctaccctttactggtacc

SEQ ID NO: 32 - DNA, 22 bp, Homo sapiens
cacaataccctttactggtacc

SEQ ID NO: 33 - DNA, 26 bp, Homo sapiens
atacttctattggtacagacaaatct

SEQ ID NO: 34 - DNA, 21 bp, Homo sapiens
cactgtctactggtaccagca

SEQ ID NO: 35 - DNA, 21 bp, Homo sapiens
cgtcatgtactggtaccagca

SEQ ID NO: 36 - DNA, 21 bp, unknown
  primer
aatgatacggcgaccaccgag

SEQ ID NO: 37 - DNA, 24 bp, Unknown
  primer
caagcagaagacggcatacgagat

SEQ ID NO: 38 - DNA, 34 bp, Unknown
  primer
agatcggaagagcacacgtctgaactccagtcac

SEQ ID NO: 39 - DNA, 34 bp, Unknown
  primer
gtgactggagttcagacgtgtgctcttccgatct

SEQ ID NO: 40 - DNA, 24 bp, Homo sapiens
cctcagtgaaggtctcctgcaagg

SEQ ID NO: 41 - DNA, 24 bp, Homo sapiens
cctcggtgaaggtctcctgcaagg

SEQ ID NO: 42 - DNA, 24 bp, Homo sapiens
cctcagtgaaggtttcctgcaagg

SEQ ID NO: 43 - DNA, 27 bp, Homo sapiens
gggctacagtgaaaatctcctgcaagg

SEQ ID NO: 44 - DNA, 26 bp, Homo sapiens
aaacccacacagaccctcacgctgac

SEQ ID NO: 45 - DNA, 26 bp, Homo sapiens
aaacccacagagaccctcacgctgac

SEQ ID NO: 46 - DNA, 26 bp, Homo sapiens
aaacccacacagaccctcacactgac

SEQ ID NO: 47 - DNA, 25 bp, Homo sapiens
ctggggggtccctgagactctcctg

SEQ ID NO: 48 - DNA, 25 bp, Homo sapiens
ctggggggtcccttagactctcctg

SEQ ID NO: 49 - DNA, 25 bp, Homo sapiens
cagggcggtccctgagactctcctg

SEQ ID NO: 50 - DNA, 25 bp, Homo sapiens
cagggccgtccctgagactctcctg

SEQ ID NO: 51 - DNA, 25 bp, Homo sapiens
ctggggggtccctgaaactctcctg

SEQ ID NO: 52 - DNA, 25 bp, Homo sapiens
ctggcaggtccctgagactctcctg

SEQ ID NO: 53 - DNA, 25 bp, Homo sapiens
ctggagggtccctgagactctcctg

SEQ ID NO: 54 - DNA, 25 bp, Homo sapiens
ctgggaggtccctgagactctcctg

SEQ ID NO: 55 - DNA, 23 bp, Homo sapiens
tgggggggccctgagactctcct

SEQ ID NO: 56 - DNA, 25 bp, Homo sapiens
cttcggagaccctgtccctcacctg

SEQ ID NO: 57 - DNA, 25 bp, Homo sapiens
cttcggacaccctgtccctcacctg

SEQ ID NO: 58 - DNA, 25 bp, Homo sapiens
cttcacagaccctgtccctcacctg

SEQ ID NO: 59 - DNA, 25 bp, Homo sapiens
cttcggagaccccgtccctcacctg

SEQ ID NO: 60 - DNA, 22 bp, Homo sapiens
cggggaccctgtccctcacctg

SEQ ID NO: 61 - DNA, 29 bp, Homo sapiens
gatctcctgtaagggttctggatacagct

SEQ ID NO: 62 - DNA, 25 bp, Homo sapiens
tcgcagaccctctcactcacctgtg

SEQ ID NO: 63 - DNA, 25 bp, Homo sapiens
tggatcaggcagtccccatcgagag

SEQ ID NO: 64 - DNA, 20 bp, Homo sapiens
gctgggtgcgccagatgccc

SEQ ID NO: 65 - DNA, 20 bp, Homo sapiens
tggatccgtcagcccccagg

SEQ ID NO: 66 - DNA, 20 bp, Homo sapiens
tggatccgtcagcccccggg

SEQ ID NO: 67 - DNA, 21 bp, Homo sapiens
gtgcgacaggcccctggacaa

SEQ ID NO: 68 - DNA, 23 bp, Homo sapiens
gggtgcgacaggccactggacaa

SEQ ID NO: 69 - DNA, 21 bp, Homo sapiens
gtgcgccaggcccccggacaa

SEQ ID NO: 70 - DNA, 23 bp, Homo sapiens
gggtgcgacaggctcgtggacaa

SEQ ID NO: 71 - DNA, 23 bp, Homo sapiens
gggtgcaacaggcccctggaaaa

SEQ ID NO: 72 - DNA, 23 bp, Homo sapiens
gggtgcgacaggctcctggaaaa

SEQ ID NO: 73 - DNA, 21 bp, Homo sapiens
gtgcgacaggcccccggacaa

SEQ ID NO: 74 - DNA, 21 bp, Homo sapiens
gtgcgacaggcccccagacaa

SEQ ID NO: 75 - DNA, 21 bp, Homo sapiens
tccgccagcccccagggaagg

SEQ ID NO: 76 - DNA, 21 bp, Homo sapiens
tccggcagcccccagggaagg

SEQ ID NO: 77 - DNA, 21 bp, Homo sapiens
tccggcagccaccagggaagg

SEQ ID NO: 78 - DNA, 21 bp, Homo sapiens
tccgccagcacccagggaagg

SEQ ID NO: 79 - DNA, 19 bp, Homo sapiens
tccggcagcccgccgggaa

SEQ ID NO: 80 - DNA, 19 bp, Homo sapiens
tccggcagccgccggggaa

SEQ ID NO: 81 - DNA, 21 bp, Homo sapiens
tccggcagcccgctgggaagg

SEQ ID NO: 82 - DNA, 21 bp, Homo sapiens
tccgccagcccctagggaagg

SEQ ID NO: 83 - DNA, 21 bp, Homo sapiens
ggtccgccaggctccagggaa

SEQ ID NO: 84 - DNA, 21 bp, Homo sapiens
gttccgccaggctccagggaa

SEQ ID NO: 85 - DNA, 21 bp, Homo sapiens
ggtccgccaggcttccgggaa

SEQ ID NO: 86 - DNA, 21 bp, Homo sapiens
ggtccgtcaagctccggggaa

SEQ ID NO: 87 - DNA, 21 bp, Homo sapiens
gatccgccaggctccagggaa

SEQ ID NO: 88 - DNA, 21 bp, Homo sapiens
ggtccgccaagctccagggaa

SEQ ID NO: 89 - DNA, 21 bp, Homo sapiens
ggtccgccaggctccaggcaa

SEQ ID NO: 90 - DNA, 21 bp, Homo sapiens
ggtccgccaggctccaggcaa

SEQ ID NO: 91 - DNA, 21 bp, Homo sapiens
ggtccgccaggctccgggcaa

SEQ ID NO: 92 - DNA, 24 bp, Homo sapiens
gggtccgtcaagctccagggaagg

SEQ ID NO: 93 - DNA, 24 bp, Homo sapiens
ctgggtccgccaagctacaggaaa

SEQ ID NO: 94 - DNA, 21 bp, Homo sapiens
ggtccgccagcctccagggaa

SEQ ID NO: 95 - DNA, 21 bp, Homo sapiens
ggtccggcaagctccagggaa

SEQ ID NO: 96 - DNA, 25 bp, Homo sapiens
ctaaaggctgaggacactgccgtgt

SEQ ID NO: 97 - DNA, 25 bp, Homo sapiens
ctctgtgactcccgaggacacggct

SEQ ID NO: 98 - DNA, 22 bp, Homo sapiens
agtggagcagcctgaaggcctc

SEQ ID NO: 99 - DNA, 25 bp, Homo sapiens
tgaccaacatggaccctgtggacac

SEQ ID NO: 100 - DNA, 25 bp, Homo sapiens
acatggagctgagcagcctgagatc

SEQ ID NO: 101 - DNA, 25 bp, Homo sapiens
acatggagctgagcaggctgagatc

SEQ ID NO: 102 - DNA, 25 bp, Homo sapiens
acatggagctgaggagcctgagatc

SEQ ID NO: 103 - DNA, 28 bp, Homo sapiens
acatggagctgaggagcctaagatctga

SEQ ID NO: 104 - DNA, 22 bp, Homo sapiens
gagctctgtgaccgccgcggac

SEQ ID NO: 105 - DNA, 23 bp, Homo sapiens
gagctctgtgaccgccgtggaca

SEQ ID NO: 106 - DNA, 25 bp, Homo sapiens
gagctctgtgaccgctgcagacacg

SEQ ID NO: 107 - DNA, 23 bp, Homo sapiens
gagctctgtgaccgctgcggaca

SEQ ID NO: 108 - DNA, 25 bp, Homo sapiens
gagctctgtgactgccgcagacacg

SEQ ID NO: 109 - DNA, 25 bp, Homo sapiens
gagctctgtgactgcagcagacacg

SEQ ID NO: 110 - DNA, 23 bp, Homo sapiens
gagctctgtgactgccgcggaca

SEQ ID NO: 111 - DNA, 22 bp, Homo sapiens
gagctctgtgaccgcggacgcg

SEQ ID NO: 112 - DNA, 21 bp, Homo sapiens
ggctctgtgaccgccgcggac

SEQ ID NO: 113 - DNA, 23 bp, Homo sapiens
gagctctgtgaccgccgcagaca

SEQ ID NO: 114 - DNA, 23 bp, Homo sapiens
gagctctgtgaccgctgacacgg

SEQ ID NO: 115 - DNA, 28 bp, Homo sapiens
caaatgaacagcctgagagccgaggaca

SEQ ID NO: 116 - DNA, 28 bp, Homo sapiens
caaatgaacagcctgaaaaccgaggaca

SEQ ID NO: 117 - DNA, 28 bp, Homo sapiens
caaatgaacagtctgaaaaccgaggaca

SEQ ID NO: 118 - DNA, 28 bp, Homo sapiens
caaatgatcagcctgaaaaccgaggaca

SEQ ID NO: 119 - DNA, 30 bp, Homo sapiens
caaatgaacagtctgagaactgaggacacc

SEQ ID NO: 120 - DNA, 28 bp, Homo sapiens
caaatgaacagtctgagagccgaggaca

SEQ ID NO: 121 - DNA, 28 bp, Homo sapiens
caaatgaacagcctgagagctgaggaca

SEQ ID NO: 122 - DNA, 28 bp, Homo sapiens
caaatgagcagcctgagagctgaggaca

SEQ ID NO: 123 - DNA, 28 bp, Homo sapiens
caaatgaacagcctgagagacgaggaca

SEQ ID NO: 124 - DNA, 28 bp, Homo sapiens
caaatgggcagcctgagagctgaggaca

SEQ ID NO: 125 - DNA, 26 bp, Homo sapiens
caaatgaacagcctgagagccgggga

SEQ ID NO: 126 - DNA, 28 bp, Homo sapiens
caaatgaacagtctgagagctgaggaca

SEQ ID NO: 127 - DNA, 28 bp, Homo sapiens
caaatgagcagtctgagagctgaggaca

SEQ ID NO: 128 - DNA, 20 bp, Homo sapiens
gccagggggaagaccgatgg

SEQ ID NO: 129 - DNA, 20 bp, Homo sapiens
gccagggggaagacggatgg

SEQ ID NO: 130 - DNA, 50 bp, Homo sapiens
aatgatacggcgaccaccgagatctgggaagacgatgggcccttggtgga

SEQ ID NO: 131 - DNA, 22 bp, Homo sapiens
gtgtgagctggatccgtcagcc

SEQ ID NO: 132 - DNA, 22 bp, Homo sapiens
gtgtgggctggatccgtcagcc

SEQ ID NO: 133 - DNA, 22 bp, Homo sapiens
gtgcgagctggatccgtcagcc

SEQ ID NO: 134 - DNA, 24 bp, Homo sapiens
gcagcctaaaggctgaggacactg

SEQ ID NO: 135 - DNA, 24 bp, Homo sapiens
gcacgctaaaggctgaggacactg

SEQ ID NO: 136 - DNA, 41 bp, Homo sapiens
  misc_feature (19)..(19): n is a, c, g, or t
acgagcctcatgcgtaganctcacctgaggagacggtgacc

SEQ ID NO: 137 - DNA, 41 bp, Homo sapiens
  misc_feature (19)..(19): n is a, c, g, or t
acgagcctcatgcgtaganctcacctgaggagacagtgacc

SEQ ID NO: 138 - DNA, 41 bp, Homo sapiens
  misc_feature (19)..(19): n is a, c, g, or t
acgagcctcatgcgtagancttacctgaagagacggtgacc

SEQ ID NO: 139 - DNA, 41 bp, Homo sapiens
  misc_feature (19)..(19): n is a, c, g, or t
acgagcctcatgcgtagancttacctgaggagacggtgacc

SEQ ID NO: 140 - DNA, 25 bp, Homo sapiens
aatgatacggcgaccaccgagatct

SEQ ID NO: 141 - DNA, 64 bp, Unknown
  primer
  misc_feature (25)..(30): n is a, c, g, or t
caagcagaagacggcatacgagatnnnnnngtgactggagttcagacgtgtgctcttccgatct

SEQ ID NO: 142 - DNA, 23 bp, mouse
tgatggctcaaacaaggagacct

SEQ ID NO: 143 - DNA, 57 bp, mouse
aatgatacggcgaccaccgagatctgaccttgggtggagtcacatttctcagatcct

SEQ ID NO: 144 - DNA, 58 bp, Homo sapiens
aatgatacggcgaccaccgagatctacactctttccctacacgagcctcatgcgtaga

SEQ ID NO: 145 - DNA, 23 bp, mouse
caaagaggtcaaatctcttcccg

SEQ ID NO: 146 - DNA, 24 bp, mouse
cttatggacaatcagactgcctca

SEQ ID NO: 147 - DNA, 28 bp, mouse
gtcatggagaagtctaaactgtttaagg

SEQ ID NO: 148 - DNA, 23 bp, mouse
gtaaacgaaacagttccaaggcg

SEQ ID NO: 149 - DNA, 26 bp, mouse
ggtgcccagtcgttttatacctgaat

SEQ ID NO: 150 - DNA, 25 bp, mouse
cccagcagattctcagtccaacagt

SEQ ID NO: 151 - DNA, 24 bp, mouse
agatatccctgatggatacaaggc

SEQ ID NO: 152 - DNA, 24 bp, mouse
agatatccctgatgggtacaaggc

SEQ ID NO: 153 - DNA, 24 bp, mouse
agatgtccctgatgggtacaaggc

SEQ ID NO: 154 - DNA, 24 bp, mouse
gataattcacagttgccctcggat

SEQ ID NO: 155 - DNA, 22 bp, mouse
gatggtggggctttcaaggatc

SEQ ID NO: 156 - DNA, 24 bp, mouse
caagctcctatagatgattcaggg

SEQ ID NO: 157 - DNA, 27 bp, mouse
ctatgataagattttgaacagggaagc

SEQ ID NO: 158 - DNA, 32 bp, mouse
gatctactattcaataactgaaaacgatcttc

SEQ ID NO: 159 - DNA, 24 bp, mouse
gcactttctactgtgaactcagca

SEQ ID NO: 160 - DNA, 25 bp, mouse
cttgatcaaatagacatggtcaagg

SEQ ID NO: 161 - DNA, 26 bp, mouse
agagattctcagctaagtgttcctcg

SEQ ID NO: 162 - DNA, 25 bp, mouse
gttcttcagcaaatagacatgactg

SEQ ID NO: 163 - DNA, 25 bp, mouse
agcgaaggagacatccctaaaggat

SEQ ID NO: 164 - DNA, 25 bp, mouse
cgagagtggattcaccaaggacaag

SEQ ID NO: 165 - DNA, 14 bp, Homo sapiens
agatcggaagagca

SEQ ID NO: 166 - DNA, 20 bp, Homo sapiens
gcctttattggtaccgacag

SEQ ID NO: 167 - DNA, 20 bp, Homo sapiens
ccctttattggtaccgacag

SEQ ID NO: 168 - DNA, 21 bp, Homo sapiens
ggctatgtattggtacaagca

SEQ ID NO: 169 - DNA, 20 bp, Homo sapiens
gtatcgacaagacccaggca

SEQ ID NO: 170 - DNA, 22 bp, Homo sapiens
atgtcctggtatcgacaagacc

SEQ ID NO: 171 - DNA, 53 bp, mouse
caaaatacagcgtttctgcactaccccaagctatactgctggcacagagaaaa

SEQ ID NO: 172 - DNA, 53 bp, mouse
caaaatacagcgtttctgcactcccccaggctatactgctggcacagagaaaa

SEQ ID NO: 173 - DNA, 53 bp, mouse
caaaatacagcgtttctgcactaccccaggctatactgctggcacagagaaaa

SEQ ID NO: 174 - DNA, 53 bp, mouse
caaaatacagcgtttctgcactcccccaagctatactgctggcacagagaaaa

SEQ ID NO: 175 - DNA, 53 bp, mouse
caaaatacagcgtttctgcacttccccaggctatactgctggcacagagaaaa

SEQ ID NO: 176 - DNA, 53 bp, mouse
caaaatacagcgtttctgcactaccccaggcaatactgctggcacagagaaaa

SEQ ID NO: 177 - DNA, 53 bp, mouse
caaaatacagcgtttctgcactcccccaggcaatactgctggcacagagaaaa

SEQ ID NO: 178 - DNA, 53 bp, mouse
caaaatacagcgtttctgcactgccccaagctatactgctggcacagagaaaa

SEQ ID NO: 179 - DNA, 53 bp, mouse
caaaatacagcgtttctgcactgccccaggctatactgctggcacagagaaaa

SEQ ID NO: 180 - DNA, 53 bp, mouse
caaaatacagcgtttctgcgctcccccatgctatactgctggcacagagaaaa

SEQ ID NO: 181 - DNA, 53 bp, Homo sapiens
ctggccccaattccatctgcctgtaaagcatgtacagtaatacacagccgtgt

SEQ ID NO: 182 - DNA, 53 bp, Homo sapiens
ctggccccagttccatttggtagtaaaacatgtacagtaatacacagccgtgt

SEQ ID NO: 183 - DNA, 53 bp, Homo sapiens
ctggccccaattccacttggtagtaaaacatgtacagtaatacacagccgtgt

SEQ ID NO: 184 - DNA, 53 bp, Homo sapiens
ctggccccaattccacttggtggtaaaacatgtacaataatagacagccgtgt

SEQ ID NO: 185 - DNA, 53 bp, Homo sapiens
ctggccccagttccatttggtagtaaaacatgtacagtaatatacagcagtgt

SEQ ID NO: 186 - DNA, 53 bp, Homo sapiens
ctggccccagttccatttggtagtaaaacatgtacagtaatatacagctgtgt

SEQ ID NO: 187 - DNA, 53 bp, Homo sapiens
ctggccccagttccatttggtagtaaaacatgtacagtaatatacagcggtgt

SEQ ID NO: 188 - DNA, 53 bp, Homo sapiens
ctggccccaattccacttggtagtaaaacatgtacagtaatagacagcagtgt

SEQ ID NO: 189 - DNA, 53 bp, Homo sapiens
ctggccccagttccatttggtagtaaaacatgtacagtaatatacggccgtgt

SEQ ID NO: 190 - DNA, 53 bp, Homo sapiens
ctggccccagttccatttggtagtaaaacatgtacagtaatatacagccgttg

SEQ ID NO: 191 - DNA, 53 bp, Homo sapiens
ctggccccagttccatctcgtagtaaaacatgtacaataatacacagccgtgt

SEQ ID NO: 192 - DNA, 53 bp, Homo sapiens
ctggccccagttccatctggtagtaaaacacgtacaataatacacagccgtgt

SEQ ID NO: 193 - protein, 17 aa, mouse
FLCASSIAWGSAETLYF

SEQ ID NO: 194 - protein, 17 aa, mouse
LYCTCSALGGSSYEQYF

SEQ ID NO: 195 - protein, 17 aa, Homo sapiens
TAVYYCTCFTGRWNWGQ

SEQ ID NO: 196 - protein, 17 aa, Homo sapiens
TAVYYCTCFTTKWNWGQ

SEQ ID NO: 197 - protein, 17 aa, Homo sapiens
TAVYYCTCFTTRWNWGQ